European Patent Application EP 4 685 232 A1, published January 28, 2026. Title: Novel Hyaluronidase Variants and Pharmaceutical Composition Comprising the Same. Applicant: Alteogen Inc. The sequence listing filed with the application follows.

SEQUENCE LISTING (70 sequences)

SEQ ID NO: 1 - protein, 435 aa, synthetic construct
  REGION 1..435: note = Synthetic Sequence
MAAHLLPICALFLTLLDMAQGFRGPLLPNRPFTTVWNANTQWCLERHGVDVDVSVFDVVANPGQTFRGPDMTIFYSSQLGTYPYYTPTGEPVFGGLPQNASLIAHLARTFQDILAAIPAPDFSGLAVIDWEAWRPRWAFNWDTKDIYRQRSRALVQAQHPDWPAPQVEAVAQDQFQGAARAWMAGTLQLGRALRPRGLWGFYGFPDCYNYDFLSPNYTGQCPSGIRAQNDQLGWLWGQSRALYPSIYMPAVLEGTGKSQMYVQHRVAEAFRVAVAAGDPNLPVLPYVQIFYDTTNHFLPLDELEHSLGESAAQGAAGVVLWVSWENTRTKESCQAIKEYMDTTLGPFILNVTSGALLCSQALCSGHGRCVRRTSHPKALLLLNPASFSIQLTPGGGPLSLRGALSLEDQAQMAVEFKCRCYPGWQAPWCERKSMW

SEQ ID NO: 2 - protein, 473 aa, synthetic construct
  REGION 1..473: note = Synthetic Sequence
MRAGPGPTVTLALVLAVSWAMELKPTAPPIFTGRPFVVAWDVPTQDCGPRLKVPLDLNAFDVQASPNEGFVNQNITIFYRDRLGLYPRFDSAGRSVHGGVPQNVSLWAHRKMLQKRVEHYIRTQESAGLAVIDWEDWRPVWVRNWQDKDVYRRLSRQLVASRHPDWPPDRIVKQAQYEFEFAAQQFMLETLRYVKAVRPRHLWGFYLFPDCYNHDYVQNWESYTGRCPDVEVARNDQLAWLWAESTALFPSVYLDETLASSRHGRNFVSFRVQEALRVARTHHANHALPVYVFTRPTYSRRLTGLSEMDLISTIGESAALGAAGVILWGDAGYTTSTETCQYLKDYLTRLLVPYVVNVSWATQYCSRAQCHGHGRCVRRNPSASTFLHLSTNSFRLVPGHAPGEPQLRPVGELSWADIDHLQTHFRCQCYLGWSGEQCQWDHRQAAGGASEAWAGSHLTSLLALAALAFTWTL

SEQ ID NO: 3 - protein, 417 aa, synthetic construct
  REGION 1..417: note = Synthetic Sequence
MTTQLGPALVLGVALCLGCGQPLPQVPERPFSVLWNVPSAHCEARFGVHLPLNALGIIANRGQHFHGQNMTIFYKNQLGLYPYFGPRGTAHNGGIPQALPLDRHLALAAYQIHHSLRPGFAGPAVLDWEEWCPLWAGNWGRRRAYQAASWAWAQQVFPDLDPQEQLYKAYTGFEQAARALMEDTLRVAQALRPHGLWGFYHYPACGNGWHSMASNYTGRCHAATLARNTQLHWLWAASSALFPSIYLPPRLPPAHHQAFVRHRLEEAFRVALVGHRHPLPVLAYVRLTHRRSGRFLSQDDLVQSIGVSAALGAAGVVLWGDLSLSSSEEECWHLHDYLVDTLGPYVINVTRAAMACSHQRCHGHGRCARRDPGQMEAFLHLWPDGSLGDWKSFSCHCYWGWAGPTCQEPRPGPKEAV

SEQ ID NO: 4 - protein, 481 aa, synthetic construct
  REGION 1..481: note = Synthetic Sequence
MKVLSEGQLKLCVVQPVHLTSWLLIFFILKSISCLKPARLPIYQRKPFIAAWNAPTDQCLIKYNLRLNLKMFPVIGSPLAKARGQNVTIFYVNRLGYYPWYTSQGVPINGGLPQNISLQVHLEKADQDINYYIPAEDFSGLAVIDWEYWRPQWARNWNSKDVYRQKSRKLISDMGKNVSATDIEYLAKVTFEESAKAFMKETIKLGIKSRPKGLWGYYLYPDCHNYNVYAPNYSGSCPEDEVLRNNELSWLWNSSAALYPSIGVWKSLGDSENILRFSKFRVHESMRISTMTSHDYALPVFVYTRLGYRDEPLFFLSKQDLVSTIGESAALGAAGIVIWGDMNLTASKANCTKVKQFVSSDLGSYIANVTRAAEVCSLHLCRNNGRCIRKMWNAPSYLHLNPASYHIEASEDGEFTVKGKASDTDLAVMADTFSCHCYQGYEGADCREIKTADGCSGVSPSPGSLMTLCLLLLASYRSIQL

SEQ ID NO: 5 - protein, 509 aa, synthetic construct
  REGION 1..509: note = Synthetic Sequence
MGVLKFKHIFFRSFVKSSGVSQIVFTFLLIPCCLTLNFRAPPVIPNVPFLWAWNAPSEFCLGKFDEPLDMSLFSFIGSPRINATGQGVTIFYVDRLGYYPYIDSITGVTVNGGIPQKISLQDHLDKAKKDITFYMPVDNLGMAVIDWEEWRPTWARNWKPKDVYKNRSIELVQQQNVQLSLTEATEKAKQEFEKAGKDFLVETIKLGKLLRPNHLWGYYLFPDCYNHHYKKPGYNGSCFNVEIKRNDDLSWLWNESTALYPSIYLNTQQSPVAATLYVRNRVREAIRVSKIPDAKSPLPVFAYTRIVFTDQVLKFLSQDELVYTFGETVALGASGIVIWGTLSIMRSMKSCLLLDNYMETILNPYIINVTLAAKMCSQVLCQEQGVCIRKNWNSSDYLHLNPDNFAIQLEKGGKFTVRGKPTLEDLEQFSEKFYCSCYSTLSCKEKADVKDTDAVDVCIADGVCIDAFLKPPMETEEPQIFYNASPSTLSATMFIVSILFLIISSVASL

SEQ ID NO: 6 - DNA, 44 bp, synthetic construct
  misc_feature 1..44: note = Synthetic Sequence
  source 1..44: mol_type = other DNA
gaatatctcgaggccaccatggcagcccacctgcttcccatctg

SEQ ID NO: 7 - DNA, 40 bp, synthetic construct
  misc_feature 1..40: note = Synthetic Sequence
  source 1..40: mol_type = other DNA
ctaattgcggccgcttatcaccacatgctcttccgctcac

SEQ ID NO: 8 - DNA, 55 bp, synthetic construct
  misc_feature 1..55: note = Synthetic Sequence
  source 1..55: mol_type = other DNA
ctaattgcggccgctcattagtggtgatggtgatgatgccacatgctcttcgctc

SEQ ID NO: 9 - DNA, 50 bp, synthetic construct
  misc_feature 1..50: note = Synthetic Sequence
  source 1..50: mol_type = other DNA
tgaaggcccagcgtgggcgccatgcatgccagtcgatgactgccagccct

SEQ ID NO: 10 - DNA, 54 bp, synthetic construct
  misc_feature 1..54: note = Synthetic Sequence
  source 1..54: mol_type = other DNA
tgggcacggatgcctgatgggcacgagccgctaccgcagtcagggaagccatag

SEQ ID NO: 11 - DNA, 46 bp, synthetic construct
  misc_feature 1..46: note = Synthetic Sequence
  source 1..46: mol_type = other DNA
taggggtaggtgcccagctgggagacatagaaaattgtcatgtcag

SEQ ID NO: 12 - DNA, 44 bp, synthetic construct
  misc_feature 1..44: note = Synthetic Sequence
  source 1..44: mol_type = other DNA
taggggtaggtgcccagctggtcgctatagaaaattgtcatgtc

SEQ ID NO: 13 - DNA, 45 bp, synthetic construct
  misc_feature 1..45: note = Synthetic Sequence
  source 1..45: mol_type = other DNA
tagtaggggtaggtgcccagccgggagctatagaaaattgtcatg

SEQ ID NO: 14 - DNA, 46 bp, synthetic construct
  misc_feature 1..46: note = Synthetic Sequence
  source 1..46: mol_type = other DNA
tgaaggcccagcgtgggcgccattcctcccagtcgatgactgccag

SEQ ID NO: 15 - DNA, 43 bp, synthetic construct
  misc_feature 1..43: note = Synthetic Sequence
  source 1..43: mol_type = other DNA
tgccggtaaatgtccttggtcttccagttgaaggcccagcgtg

SEQ ID NO: 16 - DNA, 47 bp, synthetic construct
  misc_feature 1..47: note = Synthetic Sequence
  source 1..47: mol_type = other DNA
tgagcgctgccggtaaatgtccttagggtcccagttgaaggcccagc

SEQ ID NO: 17 - DNA, 43 bp, synthetic construct
  misc_feature 1..43: note = Synthetic Sequence
  source 1..43: mol_type = other DNA
tagttggggcttagaaagtcatggttgtagcagtcagggaagc

SEQ ID NO: 18 - DNA, 46 bp, synthetic construct
  misc_feature 1..46: note = Synthetic Sequence
  source 1..46: mol_type = other DNA
tggccggtgtagttggggcttagatagtcatagttgtagcagtcag

SEQ ID NO: 19 - DNA, 44 bp, synthetic construct
  misc_feature 1..44: note = Synthetic Sequence
  source 1..44: mol_type = other DNA
tggccggtgtagttggggcttttaaagtcatagttgtagcagtc

SEQ ID NO: 20 - DNA, 46 bp, synthetic construct
  misc_feature 1..46: note = Synthetic Sequence
  source 1..46: mol_type = other DNA
atcccagcatctacatgcccgcacagctggagggcacagggaagtc

SEQ ID NO: 21 - DNA, 44 bp, synthetic construct
  misc_feature 1..44: note = Synthetic Sequence
  source 1..44: mol_type = other DNA
tctatcccagcatctacatgaacgcagtgctggagggcacaggg

SEQ ID NO: 22 - DNA, 47 bp, synthetic construct
  misc_feature 1..47: note = Synthetic Sequence
  source 1..47: mol_type = other DNA
atctgccggtgctgccctatgtccggatcttctatgacacgacaaac

SEQ ID NO: 23 - DNA, 48 bp, synthetic construct
  misc_feature 1..48: note = Synthetic Sequence
  source 1..48: mol_type = other DNA
tgccctatgtccagatcttctataccacgacaaaccactttctgcccc

SEQ ID NO: 24 - DNA, 80 bp, synthetic construct
  misc_feature 1..80: note = Synthetic Sequence
  source 1..80: mol_type = other DNA
tgggagctatagaaaattgttatgaactggccggtggcgctcttctgtgggctgcctttcacatcgaagacactgacatc

SEQ ID NO: 25 - DNA, 70 bp, synthetic construct
  misc_feature 1..70: note = Synthetic Sequence
  source 1..70: mol_type = other DNA
ttctggggcagaccaccaaacacagtgttcccagtcttttcatcgatgtaggggtaggtgcccagctggg

SEQ ID NO: 26 - DNA, 74 bp, synthetic construct
  misc_feature 1..74: note = Synthetic Sequence
  source 1..74: mol_type = other DNA
atctgccggtgctgccctatgtccagatcgtattcactgacgggtcaagcacctttctgcccctggatgagctg

SEQ ID NO: 27 - DNA, 38 bp, synthetic construct
  misc_feature 1..38: note = Synthetic Sequence
  source 1..38: mol_type = other DNA
gaatatctcgaggccaccatggcagcacatctactacc

SEQ ID NO: 28 - DNA, 60 bp, synthetic construct
  misc_feature 1..60: note = Synthetic Sequence
  source 1..60: mol_type = other DNA
ctctaattgcggccgcctatcagtggtgatggtgatgatgccacatggacttccgctcgc

SEQ ID NO: 29 - DNA, 44 bp, synthetic construct
  misc_feature 1..44: note = Synthetic Sequence
  source 1..44: mol_type = other DNA
taagggtaggttcccagttgatcggagtagaagatggtcatatc

SEQ ID NO: 30 - DNA, 43 bp, synthetic construct
  misc_feature 1..43: note = Synthetic Sequence
  source 1..43: mol_type = other DNA
tgtctgtagatgtccttggtcttccagttgaaggcccatctag

SEQ ID NO: 31 - DNA, 46 bp, synthetic construct
  misc_feature 1..46: note = Synthetic Sequence
  source 1..46: mol_type = other DNA
tatagttagggctcagaaagtcgtggttgtagcagtcagggaagcc

SEQ ID NO: 32 - DNA, 47 bp, synthetic construct
  misc_feature 1..47: note = Synthetic Sequence
  source 1..47: mol_type = other DNA
tagtaagggtaggttcccagtcgatcggagtagaagatggtcatatc

SEQ ID NO: 33 - DNA, 46 bp, synthetic construct
  misc_feature 1..46: note = Synthetic Sequence
  source 1..46: mol_type = other DNA
tgaaggcccatctaggccgccactcctcccagtcgatcacggccag

SEQ ID NO: 34 - DNA, 40 bp, synthetic construct
  misc_feature 1..40: note = Synthetic Sequence
  source 1..40: mol_type = other DNA
tgtctgtagatgtccttgggcttccagttgaaggcccatc

SEQ ID NO: 35 - DNA, 46 bp, synthetic construct
  misc_feature 1..46: note = Synthetic Sequence
  source 1..46: mol_type = other DNA
tggccggtatagttagggctcagatagtcgtggttgtagcagtcag

SEQ ID NO: 36 - DNA, 47 bp, synthetic construct
  misc_feature 1..47: note = Synthetic Sequence
  source 1..47: mol_type = other DNA
acccctccatctacatgcctgcccagctggaaggcaccggcaagagc

SEQ ID NO: 37 - DNA, 33 bp, synthetic construct
  misc_feature 1..33: note = Synthetic Sequence
  source 1..33: mol_type = other DNA
gaatatctcgaggccaccatgcctagttccgtg

SEQ ID NO: 38 - DNA, 43 bp, synthetic construct
  misc_feature 1..43: note = Synthetic Sequence
  source 1..43: mol_type = other DNA
taggcagcagggggcctctaaaagccagtgagacggggaccag

SEQ ID NO: 39 - DNA, 33 bp, synthetic construct
  misc_feature 1..33: note = Synthetic Sequence
  source 1..33: mol_type = other DNA
gaatatctcgaggccaccatgaagtgggttaca

SEQ ID NO: 40 - DNA, 43 bp, synthetic construct
  misc_feature 1..43: note = Synthetic Sequence
  source 1..43: mol_type = other DNA
taggcagcagggggcctctaaaagagtaagcagaggagaaaag

SEQ ID NO: 41 - DNA, 35 bp, synthetic construct
  misc_feature 1..35: note = Synthetic Sequence
  source 1..35: mol_type = other DNA
caatacctcgaggccaccatggctacaggctcccg

SEQ ID NO: 42 - DNA, 42 bp, synthetic construct
  misc_feature 1..42: note = Synthetic Sequence
  source 1..42: mol_type = other DNA
taggcagcagggggcctctaaaggcactgccctcttgaagcc

SEQ ID NO: 43 - DNA, 40 bp, synthetic construct
  misc_feature 1..40: note = Synthetic Sequence
  source 1..40: mol_type = other DNA
actaagctcgaggccaccatggtgagtagtgcacaatttc

SEQ ID NO: 44 - DNA, 42 bp, synthetic construct
  misc_feature 1..42: note = Synthetic Sequence
  source 1..42: mol_type = other DNA
taggcagcagggggcctctaaaacatctggtgccctggaagc

SEQ ID NO: 45 - DNA, 49 bp, synthetic construct
  misc_feature 1..49: note = Synthetic Sequence
  source 1..49: mol_type = other DNA
agccctgtacccctccatctacatgaatgccgtgctggaaggcaccggc

SEQ ID NO: 46 - DNA, 79 bp, synthetic construct
  misc_feature 1..79: note = Synthetic Sequence
  source 1..79: mol_type = other DNA
agccctgtacccctccatctacatgaatacccagcagtcacccgtcgccgcgaccctgtacgtgcagcacagagtggcc

SEQ ID NO: 47 - DNA, 51 bp, synthetic construct
  misc_feature 1..51: note = Synthetic Sequence
  source 1..51: mol_type = other DNA
tccgccgaacacaggctcgccggtagggtcgtagtaagggtaggttcccag

SEQ ID NO: 48 - protein, 435 aa, synthetic construct
  REGION 1..435: note = Synthetic Sequence
MAAHLLPICALFLTLLDMAQGFRGPLLPNRPFTTVWNANTQWCLERHGVDVDVSVFDVVANPGQTFRGPDMTIFYVSQLGTYPYYTPTGEPVFGGLPQNASLIAHLARTFQDILAAIPAPDFSGLAVIDWEAWRPRWAFNWDTKDIYRQRSRALVQAQHPDWPAPQVEAVAQDQFQGAARAWMAGTLQLGRALRPRGLWGFYGFPDCYNYDFLSPNYTGQCPSGIRAQNDQLGWLWGQSRALYPSIYMPAVLEGTGKSQMYVQHRVAEAFRVAVAAGDPNLPVLPYVQIFYDTTNHFLPLDELEHSLGESAAQGAAGVVLWVSWENTRTKESCQAIKEYMDTTLGPFILNVTSGALLCSQALCSGHGRCVRRTSHPKALLLLNPASFSIQLTPGGGPLSLRGALSLEDQAQMAVEFKCRCYPGWQAPWCERKSMW

SEQ ID NO: 49 - protein, 435 aa, synthetic construct
  REGION 1..435: note = Synthetic Sequence
MAAHLLPICALFLTLLDMAQGFRGPLLPNRPFTTVWNANTQWCLERHGVDVDVSVFDVVANPGQTFRGPDMTIFYSDQLGTYPYYTPTGEPVFGGLPQNASLIAHLARTFQDILAAIPAPDFSGLAVIDWEAWRPRWAFNWDTKDIYRQRSRALVQAQHPDWPAPQVEAVAQDQFQGAARAWMAGTLQLGRALRPRGLWGFYGFPDCYNYDFLSPNYTGQCPSGIRAQNDQLGWLWGQSRALYPSIYMPAVLEGTGKSQMYVQHRVAEAFRVAVAAGDPNLPVLPYVQIFYDTTNHFLPLDELEHSLGESAAQGAAGVVLWVSWENTRTKESCQAIKEYMDTTLGPFILNVTSGALLCSQALCSGHGRCVRRTSHPKALLLLNPASFSIQLTPGGGPLSLRGALSLEDQAQMAVEFKCRCYPGWQAPWCERKSMW

SEQ ID NO: 50 - protein, 435 aa, synthetic construct
  REGION 1..435: note = Synthetic Sequence
MAAHLLPICALFLTLLDMAQGFRGPLLPNRPFTTVWNANTQWCLERHGVDVDVSVFDVVANPGQTFRGPDMTIFYSSRLGTYPYYTPTGEPVFGGLPQNASLIAHLARTFQDILAAIPAPDFSGLAVIDWEAWRPRWAFNWDTKDIYRQRSRALVQAQHPDWPAPQVEAVAQDQFQGAARAWMAGTLQLGRALRPRGLWGFYGFPDCYNYDFLSPNYTGQCPSGIRAQNDQLGWLWGQSRALYPSIYMPAVLEGTGKSQMYVQHRVAEAFRVAVAAGDPNLPVLPYVQIFYDTTNHFLPLDELEHSLGESAAQGAAGVVLWVSWENTRTKESCQAIKEYMDTTLGPFILNVTSGALLCSQALCSGHGRCVRRTSHPKALLLLNPASFSIQLTPGGGPLSLRGALSLEDQAQMAVEFKCRCYPGWQAPWCERKSMW

SEQ ID NO: 51 - protein, 435 aa, synthetic construct
  REGION 1..435: note = Synthetic Sequence
MAAHLLPICALFLTLLDMAQGFRGPLLPNRPFTTVWNANTQWCLERHGVDVDVSVFDVVANPGQTFRGPDMTIFYSSQLGTYPYYTPTGEPVFGGLPQNASLIAHLARTFQDILAAIPAPDFSGLAVIDWEEWRPRWAFNWDTKDIYRQRSRALVQAQHPDWPAPQVEAVAQDQFQGAARAWMAGTLQLGRALRPRGLWGFYGFPDCYNYDFLSPNYTGQCPSGIRAQNDQLGWLWGQSRALYPSIYMPAVLEGTGKSQMYVQHRVAEAFRVAVAAGDPNLPVLPYVQIFYDTTNHFLPLDELEHSLGESAAQGAAGVVLWVSWENTRTKESCQAIKEYMDTTLGPFILNVTSGALLCSQALCSGHGRCVRRTSHPKALLLLNPASFSIQLTPGGGPLSLRGALSLEDQAQMAVEFKCRCYPGWQAPWCERKSMW

SEQ ID NO: 52 - protein, 435 aa, synthetic construct
  REGION 1..435: note = Synthetic Sequence
MAAHLLPICALFLTLLDMAQGFRGPLLPNRPFTTVWNANTQWCLERHGVDVDVSVFDVVANPGQTFRGPDMTIFYSSQLGTYPYYTPTGEPVFGGLPQNASLIAHLARTFQDILAAIPAPDFSGLAVIDWEAWRPRWAFNWKTKDIYRQRSRALVQAQHPDWPAPQVEAVAQDQFQGAARAWMAGTLQLGRALRPRGLWGFYGFPDCYNYDFLSPNYTGQCPSGIRAQNDQLGWLWGQSRALYPSIYMPAVLEGTGKSQMYVQHRVAEAFRVAVAAGDPNLPVLPYVQIFYDTTNHFLPLDELEHSLGESAAQGAAGVVLWVSWENTRTKESCQAIKEYMDTTLGPFILNVTSGALLCSQALCSGHGRCVRRTSHPKALLLLNPASFSIQLTPGGGPLSLRGALSLEDQAQMAVEFKCRCYPGWQAPWCERKSMW

SEQ ID NO: 53 - protein, 435 aa, synthetic construct
  REGION 1..435: note = Synthetic Sequence
MAAHLLPICALFLTLLDMAQGFRGPLLPNRPFTTVWNANTQWCLERHGVDVDVSVFDVVANPGQTFRGPDMTIFYSSQLGTYPYYTPTGEPVFGGLPQNASLIAHLARTFQDILAAIPAPDFSGLAVIDWEAWRPRWAFNWDPKDIYRQRSRALVQAQHPDWPAPQVEAVAQDQFQGAARAWMAGTLQLGRALRPRGLWGFYGFPDCYNYDFLSPNYTGQCPSGIRAQNDQLGWLWGQSRALYPSIYMPAVLEGTGKSQMYVQHRVAEAFRVAVAAGDPNLPVLPYVQIFYDTTNHFLPLDELEHSLGESAAQGAAGVVLWVSWENTRTKESCQAIKEYMDTTLGPFILNVTSGALLCSQALCSGHGRCVRRTSHPKALLLLNPASFSIQLTPGGGPLSLRGALSLEDQAQMAVEFKCRCYPGWQAPWCERKSMW

SEQ ID NO: 54 - protein, 435 aa, synthetic construct
  REGION 1..435: note = Synthetic Sequence
MAAHLLPICALFLTLLDMAQGFRGPLLPNRPFTTVWNANTQWCLERHGVDVDVSVFDVVANPGQTFRGPDMTIFYSSQLGTYPYYTPTGEPVFGGLPQNASLIAHLARTFQDILAAIPAPDFSGLAVIDWEAWRPRWAFNWDTKDIYRQRSRALVQAQHPDWPAPQVEAVAQDQFQGAARAWMAGTLQLGRALRPRGLWGFYGFPDCYNHDFLSPNYTGQCPSGIRAQNDQLGWLWGQSRALYPSIYMPAVLEGTGKSQMYVQHRVAEAFRVAVAAGDPNLPVLPYVQIFYDTTNHFLPLDELEHSLGESAAQGAAGVVLWVSWENTRTKESCQAIKEYMDTTLGPFILNVTSGALLCSQALCSGHGRCVRRTSHPKALLLLNPASFSIQLTPGGGPLSLRGALSLEDQAQMAVEFKCRCYPGWQAPWCERKSMW

SEQ ID NO: 55 - protein, 435 aa, synthetic construct
  REGION 1..435: note = Synthetic Sequence
MAAHLLPICALFLTLLDMAQGFRGPLLPNRPFTTVWNANTQWCLERHGVDVDVSVFDVVANPGQTFRGPDMTIFYSSQLGTYPYYTPTGEPVFGGLPQNASLIAHLARTFQDILAAIPAPDFSGLAVIDWEAWRPRWAFNWDTKDIYRQRSRALVQAQHPDWPAPQVEAVAQDQFQGAARAWMAGTLQLGRALRPRGLWGFYGFPDCYNYDYLSPNYTGQCPSGIRAQNDQLGWLWGQSRALYPSIYMPAVLEGTGKSQMYVQHRVAEAFRVAVAAGDPNLPVLPYVQIFYDTTNHFLPLDELEHSLGESAAQGAAGVVLWVSWENTRTKESCQAIKEYMDTTLGPFILNVTSGALLCSQALCSGHGRCVRRTSHPKALLLLNPASFSIQLTPGGGPLSLRGALSLEDQAQMAVEFKCRCYPGWQAPWCERKSMW

SEQ ID NO: 56 - protein, 435 aa, synthetic construct
  REGION 1..435: note = Synthetic Sequence
MAAHLLPICALFLTLLDMAQGFRGPLLPNRPFTTVWNANTQWCLERHGVDVDVSVFDVVANPGQTFRGPDMTIFYSSQLGTYPYYTPTGEPVFGGLPQNASLIAHLARTFQDILAAIPAPDFSGLAVIDWEAWRPRWAFNWDTKDIYRQRSRALVQAQHPDWPAPQVEAVAQDQFQGAARAWMAGTLQLGRALRPRGLWGFYGFPDCYNYDFKSPNYTGQCPSGIRAQNDQLGWLWGQSRALYPSIYMPAVLEGTGKSQMYVQHRVAEAFRVAVAAGDPNLPVLPYVQIFYDTTNHFLPLDELEHSLGESAAQGAAGVVLWVSWENTRTKESCQAIKEYMDTTLGPFILNVTSGALLCSQALCSGHGRCVRRTSHPKALLLLNPASFSIQLTPGGGPLSLRGALSLEDQAQMAVEFKCRCYPGWQAPWCERKSMW

SEQ ID NO: 57 - protein, 435 aa, synthetic construct
  REGION 1..435: note = Synthetic Sequence
MAAHLLPICALFLTLLDMAQGFRGPLLPNRPFTTVWNANTQWCLERHGVDVDVSVFDVVANPGQTFRGPDMTIFYSSQLGTYPYYTPTGEPVFGGLPQNASLIAHLARTFQDILAAIPAPDFSGLAVIDWEAWRPRWAFNWDTKDIYRQRSRALVQAQHPDWPAPQVEAVAQDQFQGAARAWMAGTLQLGRALRPRGLWGFYGFPDCYNYDFLSPNYTGQCPSGIRAQNDQLGWLWGQSRALYPSIYMPAQLEGTGKSQMYVQHRVAEAFRVAVAAGDPNLPVLPYVQIFYDTTNHFLPLDELEHSLGESAAQGAAGVVLWVSWENTRTKESCQAIKEYMDTTLGPFILNVTSGALLCSQALCSGHGRCVRRTSHPKALLLLNPASFSIQLTPGGGPLSLRGALSLEDQAQMAVEFKCRCYPGWQAPWCERKSMW

SEQ ID NO: 58 - protein, 435 aa, synthetic construct
  REGION 1..435: note = Synthetic Sequence
MAAHLLPICALFLTLLDMAQGFRGPLLPNRPFTTVWNANTQWCLERHGVDVDVSVFDVVANPGQTFRGPDMTIFYSSQLGTYPYYTPTGEPVFGGLPQNASLIAHLARTFQDILAAIPAPDFSGLAVIDWEAWRPRWAFNWDTKDIYRQRSRALVQAQHPDWPAPQVEAVAQDQFQGAARAWMAGTLQLGRALRPRGLWGFYGFPDCYNYDFLSPNYTGQCPSGIRAQNDQLGWLWGQSRALYPSIYMNAVLEGTGKSQMYVQHRVAEAFRVAVAAGDPNLPVLPYVQIFYDTTNHFLPLDELEHSLGESAAQGAAGVVLWVSWENTRTKESCQAIKEYMDTTLGPFILNVTSGALLCSQALCSGHGRCVRRTSHPKALLLLNPASFSIQLTPGGGPLSLRGALSLEDQAQMAVEFKCRCYPGWQAPWCERKSMW

SEQ ID NO: 59 - protein, 435 aa, synthetic construct
  REGION 1..435: note = Synthetic Sequence
MAAHLLPICALFLTLLDMAQGFRGPLLPNRPFTTVWNANTQWCLERHGVDVDVSVFDVVANPGQTFRGPDMTIFYSSQLGTYPYYTPTGEPVFGGLPQNASLIAHLARTFQDILAAIPAPDFSGLAVIDWEAWRPRWAFNWDTKDIYRQRSRALVQAQHPDWPAPQVEAVAQDQFQGAARAWMAGTLQLGRALRPRGLWGFYGFPDCYNYDFLSPNYTGQCPSGIRAQNDQLGWLWGQSRALYPSIYMPAVLEGTGKSQMYVQHRVAEAFRVAVAAGDPNLPVLPYVRIFYDTTNHFLPLDELEHSLGESAAQGAAGVVLWVSWENTRTKESCQAIKEYMDTTLGPFILNVTSGALLCSQALCSGHGRCVRRTSHPKALLLLNPASFSIQLTPGGGPLSLRGALSLEDQAQMAVEFKCRCYPGWQAPWCERKSMW

SEQ ID NO: 60 - protein, 435 aa, synthetic construct
  REGION 1..435: note = Synthetic Sequence
MAAHLLPICALFLTLLDMAQGFRGPLLPNRPFTTVWNANTQWCLERHGVDVDVSVFDVVANPGQTFRGPDMTIFYSSQLGTYPYYTPTGEPVFGGLPQNASLIAHLARTFQDILAAIPAPDFSGLAVIDWEAWRPRWAFNWDTKDIYRQRSRALVQAQHPDWPAPQVEAVAQDQFQGAARAWMAGTLQLGRALRPRGLWGFYGFPDCYNYDFLSPNYTGQCPSGIRAQNDQLGWLWGQSRALYPSIYMPAVLEGTGKSQMYVQHRVAEAFRVAVAAGDPNLPVLPYVQIFYTTTNHFLPLDELEHSLGESAAQGAAGVVLWVSWENTRTKESCQAIKEYMDTTLGPFILNVTSGALLCSQALCSGHGRCVRRTSHPKALLLLNPASFSIQLTPGGGPLSLRGALSLEDQAQMAVEFKCRCYPGWQAPWCERKSMW

SEQ ID NO: 61 - protein, 435 aa, synthetic construct
  REGION 1..435: note = Synthetic Sequence
MAAHLLPICALFLTLLDMAQGFRGPLLPNRPFTTVWNANTQWCLERHGVDVDVSVFDVVANPGQTFRGPDMTIFYSDQLGTYPYYTPTGEPVFGGLPQNASLIAHLARTFQDILAAIPAPDFSGLAVIDWEAWRPRWAFNWKTKDIYRQRSRALVQAQHPDWPAPQVEAVAQDQFQGAARAWMAGTLQLGRALRPRGLWGFYGFPDCYNHDFLSPNYTGQCPSGIRAQNDQLGWLWGQSRALYPSIYMPAVLEGTGKSQMYVQHRVAEAFRVAVAAGDPNLPVLPYVQIFYDTTNHFLPLDELEHSLGESAAQGAAGVVLWVSWENTRTKESCQAIKEYMDTTLGPFILNVTSGALLCSQALCSGHGRCVRRTSHPKALLLLNPASFSIQLTPGGGPLSLRGALSLEDQAQMAVEFKCRCYPGWQAPWCERKSMW

SEQ ID NO: 62 - protein, 435 aa, synthetic construct
  REGION 1..435: note = Synthetic Sequence
MAAHLLPICALFLTLLDMAQGFRGPLLPNRPFTTVWNANTQWCLERHGVDVDVSVFDVVANPGQTFRGPDMTIFYSDRLGTYPYYTPTGEPVFGGLPQNASLIAHLARTFQDILAAIPAPDFSGLAVIDWEAWRPRWAFNWKTKDIYRQRSRALVQAQHPDWPAPQVEAVAQDQFQGAARAWMAGTLQLGRALRPRGLWGFYGFPDCYNHDFLSPNYTGQCPSGIRAQNDQLGWLWGQSRALYPSIYMPAVLEGTGKSQMYVQHRVAEAFRVAVAAGDPNLPVLPYVQIFYDTTNHFLPLDELEHSLGESAAQGAAGVVLWVSWENTRTKESCQAIKEYMDTTLGPFILNVTSGALLCSQALCSGHGRCVRRTSHPKALLLLNPASFSIQLTPGGGPLSLRGALSLEDQAQMAVEFKCRCYPGWQAPWCERKSMW

SEQ ID NO: 63 - protein, 435 aa, synthetic construct
  REGION 1..435: note = Synthetic Sequence
MAAHLLPICALFLTLLDMAQGFRGPLLPNRPFTTVWNANTQWCLERHGVDVDVSVFDVVANPGQTFRGPDMTIFYSDQLGTYPYYTPTGEPVFGGLPQNASLIAHLARTFQDILAAIPAPDFSGLAVIDWEEWRPRWAFNWKTKDIYRQRSRALVQAQHPDWPAPQVEAVAQDQFQGAARAWMAGTLQLGRALRPRGLWGFYGFPDCYNHDFLSPNYTGQCPSGIRAQNDQLGWLWGQSRALYPSIYMPAVLEGTGKSQMYVQHRVAEAFRVAVAAGDPNLPVLPYVQIFYDTTNHFLPLDELEHSLGESAAQGAAGVVLWVSWENTRTKESCQAIKEYMDTTLGPFILNVTSGALLCSQALCSGHGRCVRRTSHPKALLLLNPASFSIQLTPGGGPLSLRGALSLEDQAQMAVEFKCRCYPGWQAPWCERKSMW

SEQ ID NO: 64 - protein, 435 aa, synthetic construct
  REGION 1..435: note = Synthetic Sequence
MAAHLLPICALFLTLLDMAQGFRGPLLPNRPFTTVWNANTQWCLERHGVDVDVSVFDVVANPGQTFRGPDMTIFYSDQLGTYPYYTPTGEPVFGGLPQNASLIAHLARTFQDILAAIPAPDFSGLAVIDWEAWRPRWAFNWKPKDIYRQRSRALVQAQHPDWPAPQVEAVAQDQFQGAARAWMAGTLQLGRALRPRGLWGFYGFPDCYNHDFLSPNYTGQCPSGIRAQNDQLGWLWGQSRALYPSIYMPAVLEGTGKSQMYVQHRVAEAFRVAVAAGDPNLPVLPYVQIFYDTTNHFLPLDELEHSLGESAAQGAAGVVLWVSWENTRTKESCQAIKEYMDTTLGPFILNVTSGALLCSQALCSGHGRCVRRTSHPKALLLLNPASFSIQLTPGGGPLSLRGALSLEDQAQMAVEFKCRCYPGWQAPWCERKSMW

SEQ ID NO: 65 - protein, 435 aa, synthetic construct
  REGION 1..435: note = Synthetic Sequence
MAAHLLPICALFLTLLDMAQGFRGPLLPNRPFTTVWNANTQWCLERHGVDVDVSVFDVVANPGQTFRGPDMTIFYSDQLGTYPYYTPTGEPVFGGLPQNASLIAHLARTFQDILAAIPAPDFSGLAVIDWEAWRPRWAFNWKTKDIYRQRSRALVQAQHPDWPAPQVEAVAQDQFQGAARAWMAGTLQLGRALRPRGLWGFYGFPDCYNHDYLSPNYTGQCPSGIRAQNDQLGWLWGQSRALYPSIYMPAVLEGTGKSQMYVQHRVAEAFRVAVAAGDPNLPVLPYVQIFYDTTNHFLPLDELEHSLGESAAQGAAGVVLWVSWENTRTKESCQAIKEYMDTTLGPFILNVTSGALLCSQALCSGHGRCVRRTSHPKALLLLNPASFSIQLTPGGGPLSLRGALSLEDQAQMAVEFKCRCYPGWQAPWCERKSMW

SEQ ID NO: 66 - protein, 435 aa, synthetic construct
  REGION 1..435: note = Synthetic Sequence
MAAHLLPICALFLTLLDMAQGFRGPLLPNRPFTTVWNANTQWCLERHGVDVDVSVFDVVANPGQTFRGPDMTIFYSDQLGTYPYYTPTGEPVFGGLPQNASLIAHLARTFQDILAAIPAPDFSGLAVIDWEAWRPRWAFNWKTKDIYRQRSRALVQAQHPDWPAPQVEAVAQDQFQGAARAWMAGTLQLGRALRPRGLWGFYGFPDCYNHDFLSPNYTGQCPSGIRAQNDQLGWLWGQSRALYPSIYMPAQLEGTGKSQMYVQHRVAEAFRVAVAAGDPNLPVLPYVQIFYDTTNHFLPLDELEHSLGESAAQGAAGVVLWVSWENTRTKESCQAIKEYMDTTLGPFILNVTSGALLCSQALCSGHGRCVRRTSHPKALLLLNPASFSIQLTPGGGPLSLRGALSLEDQAQMAVEFKCRCYPGWQAPWCERKSMW

SEQ ID NO: 67 - protein, 435 aa, synthetic construct
  REGION 1..435: note = Synthetic Sequence
MAAHLLPICALFLTLLDMAQGFRGPLLPNRPFTTVWNANTQWCLERHGVDVDVSVFDVVANPGQTFRGPDMTIFYSSQLGTYPYYTPTGEPVFGGLPQNASLIAHLARTFQDILAAIPAPDFSGLAVIDWEAWRPRWAFNWKTKDIYRQRSRALVQAQHPDWPAPQVEAVAQDQFQGAARAWMAGTLQLGRALRPRGLWGFYGFPDCYNHDFLSPNYTGQCPSGIRAQNDQLGWLWGQSRALYPSIYMNAVLEGTGKSQMYVQHRVAEAFRVAVAAGDPNLPVLPYVQIFYDTTNHFLPLDELEHSLGESAAQGAAGVVLWVSWENTRTKESCQAIKEYMDTTLGPFILNVTSGALLCSQALCSGHGRCVRRTSHPKALLLLNPASFSIQLTPGGGPLSLRGALSLEDQAQMAVEFKCRCYPGWQAPWCERKSMW

SEQ ID NO: 68 - protein, 435 aa, synthetic construct
  REGION 1..435: note = Synthetic Sequence
MAAHLLPICALFLTLLDMAQGFRGPLLPNRPFTTVWNANTQWCLERHGVDVDVSVFDVVANPGQTFRGPDMTIFYSSQLGTYPYYTPTGEPVFGGLPQNASLIAHLARTFQDILAAIPAPDFSGLAVIDWEAWRPRWAFNWKTKDIYRQRSRALVQAQHPDWPAPQVEAVAQDQFQGAARAWMAGTLQLGRALRPRGLWGFYGFPDCYNHDFLSPNYTGQCPSGIRAQNDQLGWLWGQSRALYPSIYMPAVLEGTGKSQMYVQHRVAEAFRVAVAAGDPNLPVLPYVQIFYDTTNHFLPLDELEHSLGESAAQGAAGVVLWVSWENTRTKESCQAIKEYMDTTLGPFILNVTSGALLCSQALCSGHGRCVRRTSHPKALLLLNPASFSIQLTPGGGPLSLRGALSLEDQAQMAVEFKCRCYPGWQAPWCERKSMW

SEQ ID NO: 69 - protein, 435 aa, synthetic construct
  REGION 1..435: note = Synthetic Sequence
MAAHLLPICALFLTLLDMAQGFRGPLLPNRPFTTVWNANTQWCLERHGVDVDVSVFDVVANPGQTFRGPDMTIFYSDQLGTYPYYTPTGEPVFGGLPQNASLIAHLARTFQDILAAIPAPDFSGLAVIDWEEWRPRWAFNWDTKDIYRQRSRALVQAQHPDWPAPQVEAVAQDQFQGAARAWMAGTLQLGRALRPRGLWGFYGFPDCYNYDFLSPNYTGQCPSGIRAQNDQLGWLWGQSRALYPSIYMPAVLEGTGKSQMYVQHRVAEAFRVAVAAGDPNLPVLPYVQIFYDTTNHFLPLDELEHSLGESAAQGAAGVVLWVSWENTRTKESCQAIKEYMDTTLGPFILNVTSGALLCSQALCSGHGRCVRRTSHPKALLLLNPASFSIQLTPGGGPLSLRGALSLEDQAQMAVEFKCRCYPGWQAPWCERKSMW

SEQ ID NO: 70 - protein, 435 aa, synthetic construct
  REGION 1..435: note = Synthetic Sequence
MAAHLLPICALFLTLLDMAQGFRGPLLPNRPFTTVWNANTQWCLERHGVDVDVSVFDVVANPGQTFRGPDMTIFYSDQLGTYPYYDPTGEPVFGGLPQNASLIAHLARTFQDILAAIPAPDFSGLAVIDWEAWRPRWAFNWDTKDIYRQRSRALVQAQHPDWPAPQVEAVAQDQFQGAARAWMAGTLQLGRALRPRGLWGFYGFPDCYNYDFLSPNYTGQCPSGIRAQNDQLGWLWGQSRALYPSIYMPAVLEGTGKSQMYVQHRVAEAFRVAVAAGDPNLPVLPYVQIFYDTTNHFLPLDELEHSLGESAAQGAAGVVLWVSWENTRTKESCQAIKEYMDTTLGPFILNVTSGALLCSQALCSGHGRCVRRTSHPKALLLLNPASFSIQLTPGGGPLSLRGALSLEDQAQMAVEFKCRCYPGWQAPWCERKSMW